European Patent Specification EP 4 076 662 B1, published January 31, 2024. Title: PYRAZOLYL DERIVATIVES USEFUL AS ANTI-CANCER AGENTS. Applicant: NOVARTIS AG. The sequence listing filed with the application follows.

SEQUENCE LISTING (1 sequence)

SEQ ID NO: 1 - DNA, 5128 bp, Artificial Sequence
  source: /note="Description of Artificial Sequence: Synthetic polynucleotide"
atgcgtccggcgtagaggatcgagatcgatctcgatcccgcgaaattaatacgactcactataggggaattgtgagcggataacaattcccctctagaaataattttgtttaactttaagaaggagatatacatatgaaaacacatcatcatcatcatcatggtggcggcagtggcggtggctcaggcggtggttctctcgaggttctgttccagggtccgggtttgaacgacatcttcgaagctcagaagatcgaatggcacgagggtggcggtagtggtggtggctctatgactgaatacaagctggttgttgttggtgcttgtggcgttggtaagagcgcactgaccatccagctcattcagaatcacttcgtggacgagtacgacccgaccatcgaagattcttaccgtaaacaggtggttattgatggcgaaacctgtctgctggatattctggacactgctggtcaggaagagtactccgctatgcgtgatcagtacatgcgtactggtgaaggtttcctctgcgtgttcgctatcaacaacaccaagtccttcgaagatatccaccattaccgtgaacagatcaaacgtgtgaaggacagcgaagacgtgccaatggttctggtgggcaacaaatgtgatctcccgagccgtaccgttgacaccaaacaggcacaagacctggcacgttcctacggcatcccattcattgaaactagcgcgaagactcgtcagggtgtggacgacgcattctacactctggtgcgtgaaattcgcaagcacaaagagaaataatggtaccgaattcgcggccgcctgcagcctaggctgctaaacaaagcccgaaaggaagctgagttggctgctgccaccgctgagcaataactagcataaccccttggggcctctaaacgggtcttgaggggttttttgctgaaaggaggaactatatccggattggcgaatgggacgcgccctgtagcggcgcattaagtgcagcgtcaaaagggcgacacaaaatttattctaaatgcataataaatactgataacatcttatagtttgtattatattttgtattatcgttgacatgtataattttgatatcaaaaactgattttccctttattattttcgagatttattttcttaattctctttaacaaactagaaatattgtatatacaaaaaatcataaataatagatgaatagtttaattataggtgttcatcaatcgaaaaagcaacgtatcttatttaaagtgcgttgcttttttctcatttataaggttaaataattctcatatatcaagcaaagtgacaggcgcccttaaatattctgacaaatgctctttccctaaactccccccataaaaaaacccgccgaagcgggtttttacgttatttgcggattaacgattactcgttatcagaaccgcccagggggcccgagcttaagactggccgtcgttttacaacacagaaagagtttgtagaaacgcaaaaaggccatccgtcaggggccttctgcttagtttgatgcctggcagttccctactctcgccttccgcttcctcgctcactgactcgctgcgctcggtcgttcggctgcggcgagcggtatcagctcactcaaaggcggtaatacggttatccacagaatcaggggataacgcaggaaagaacatgtgagcaaaaggccagcaaaaggccaggaaccgtaaaaaggccgcgttgctggcgtttttccataggctccgcccccctgacgagcatcacaaaaatcgacgctcaagtcagaggtggcgaaacccgacaggactataaagataccaggcgtttccccctggaagctccctcgtgcgctctcctgttccgaccctgccgcttaccggatacctgtccgcctttctcccttcgggaagcgtggcgctttctcatagctcacgctgtaggtatctcagttcggtgtaggtcgttcgctccaagctgggctgtgtgcacgaaccccccgttcagcccgaccgctgcgccttatccggtaactatcgtcttgagtccaacccggtaagacacgacttatcgccactggcagcagccactggtaacaggattagcagagcgaggtatgtaggcggtgctacagagttcttgaagtggtgggctaactacggctacactagaagaacagtatttggtatctgcgctctgctgaagccagttaccttcggaaaaagagttggtagctcttgatccggcaaacaaaccaccgctggtagcggtggtttttttgtttgcaagcagcagattacgcgcagaaaaaaaggatctcaagaagatcctttgatcttttctacggggtctgacgctcagtggaacgacgcgcgcgtaactcacgttaagggattttggtcatgagcttgcgccgtcccgtcaagtcagcgtaatgctctgcttttagaaaaactcatcgagcatcaaatgaaactgcaatttattcatatcaggattatcaataccatatttttgaaaaagccgtttctgtaatgaaggagaaaactcaccgaggcagttccataggatggcaagatcctggtatcggtctgcgattccgactcgtccaacatcaatacaacctattaatttcccctcgtcaaaaataaggttatcaagtgagaaatcaccatgagtgacgactgaatccggtgagaatggcaaaagtttatgcatttctttccagacttgttcaacaggccagccattacgctcgtcatcaaaatcactcgcatcaaccaaaccgttattcattcgtgattgcgcctgagcgaggcgaaatacgcgatcgctgttaaaaggacaattacaaacaggaatcgagtgcaaccggcgcaggaacactgccagcgcatcaacaatattttcacctgaatcaggatattcttctaatacctggaacgctgtttttccggggatcgcagtggtgagtaaccatgcatcatcaggagtacggataaaatgcttgatggtcggaagtggcataaattccgtcagccagtttagtctgaccatctcatctgtaacatcattggcaacgctacctttgccatgtttcagaaacaactctggcgcatcgggcttcccatacaagcgatagattgtcgcacctgattgcccgacattatcgcgagcccatttatacccatataaatcagcatccatgttggaatttaatcgcggcctcgacgtttcccgttgaatatggctcatattcttcctttttcaatattattgaagcatttatcagggttattgtctcatgagcggatacatatttgaatgtatttagaaaaataaacaaataggggtcagtgttacaaccaattaaccaattctgaacattatcgcgagcccatttatacctgaatatggctcataacaccccttgtttgcctggcggcagtagcgcggtggtcccacctgaccccatgccgaactcagaagtgaaacgccgtagcgccgatggtagtgtggggactccccatgcgagagtagggaactgccaggcatcaaataaaacgaaaggctcagtcgaaagactgggcctttcgcccgggctaattagggggtgtcgcccttcgctgaagaattgatcccggtgcctaatgagtgagctaacttacattaattgcgttgcgctcactgcccgctttccagtcgggaaacctgtcgtgccagctgcattaatgaatcggccaacgcgcggggagaggcggtttgcgtattgggcgccagggtggtttttcttttcaccagtgacacgggcaacagctgattgcccttcaccgcctggccctgagagagttgcagcaagcggtccacgctggtttgccccagcaggcgaaaatcctgtttgatggtggttaacggcgggatataacatgagctgtcttcggtatcgtcgtatcccactaccgagatgtccgcaccaacgcgcagcccggactcggtaatggcgcgcattgcgcccagcgccatctgatcgttggcaaccagcatcgcagtgggaacgatgccctcattcagcatttgcatggtttgttgaaaaccggacatggcactccagtcgccttcccgttccgctatcggctgaatttgattgcgagtgagatatttatgccagccagccagacgcagacgcgccgagacagaacttaatgggcccgctaacagcgcgatttgctggtgacccaatgcgaccagatgctccacgcccagtcgcgtaccgtcttcatgggagaaaataatactgttgatgggtgtctggtcagagacatcaagaaataacgccggaacattagtgcaggcagcttccacagcaatggcatcctggtcatccagcggatagttaatgatcagcccactgacgcgttgcgcgagaagattgtgcaccgccgctttacaggcttcgacgccgcttcgttctaccatcgacaccaccacgctggcacccagttgatcggcgcgagatttaatcgccgcgacaatttgcgacggcgcgtgcagggccagactggaggtggcaacgccaatcagcaacgactgtttgcccgccagttgttgtgccacgcggttgggaatgtaattcagctccgccatcgccgcttccactttttcccgcgttttcgcagaaacgtggctggcctggttcaccacgcgggaaacggtctgataagagacaccggcatactctgcgacatcgtataacgttactggtttcacattcaccaccctgaattgactctcttccgggcgctatcatgccataccgcgaaaggttttgcgccattcgatggtgtccgggatctcgacgctctcccttatgcgactcctgcattaggaagcagcccagtagtaggttgaggccgttgagcaccgccgccgcaaggaatggtgcatgcaaggagatggcgcccaacagtcccccggccacggggcctgccaccatacccacgccgaaacaagcgctcatgagcccgaagtggcgagcccgatcttccccatcggtgatgtcggcgatataggcgccagcaaccgcacctgtggcgccggtgatgccggccacg